European Patent Specification EP 3 956 464 B1, published December 6, 2023. Title: IN VITRO METHOD FOR THE DIAGNOSIS OR PROGNOSIS OF COLORECTAL CANCER OR A PRE-CANCEROUS STAGE THEREOF. Applicant: SERVIZO GALEGO DE SAÚDE FUNDACIÓN INSTITUTO DE INVESTIGACIÓN SANITARIA DE SANTIAGO DE COMPOSTELA. The sequence listing filed with the application follows.

SEQUENCE LISTING (9 sequences)

SEQ ID NO: 1 - DNA, 27 bp, Artificial sequence
  Artificial sequence
ggggaggygataggtttggttttagtt

SEQ ID NO: 2 - DNA, 23 bp, Artificial sequence
  Artificial sequence
acacaccaaaaatcttttctacc

SEQ ID NO: 3 - DNA, 22 bp, Artificial sequence
  Artificial sequence
gataggtttggttttagttata

SEQ ID NO: 4 - DNA, 20 bp, Artificial sequence
  Artificial sequence
tacggttttgggtcgttagc

SEQ ID NO: 5 - DNA, 20 bp, Artificial sequence
  Artificial sequence
cgaaaccaacacgaacgata

SEQ ID NO: 6 - DNA, 23 bp, Artificial sequence
  Artificial sequence
gtatggttttgggttgttagtgg

SEQ ID NO: 7 - DNA, 23 bp, Artificial sequence
  Artificial sequence
ccaaaaccaacacaaacaataac

SEQ ID NO: 8 - DNA, 20 bp, Artificial sequence
  Artificial sequence
taacgttgcgttatttgggc

SEQ ID NO: 9 - DNA, 27 bp, Artificial sequence
  Artificial sequence
ttagttataatgttgtgttatttgggt